European Patent Application EP 4 549 585 A1, published May 7, 2025. Title: DIAGNOSTIC AND THERAPEUTIC AGENT FOR SPORADIC ALZHEIMER'S DISEASE. Applicant: エーザイ・アール・アンド・ディー・マネジメント株式会社. Application JP. The sequence listing filed with the application follows.

SEQUENCE LISTING (30 sequences)

SEQ ID NO: 1 - protein, 480 aa, Homo sapiens
MKRSVAVWLLVGLSLGVPQFGKGDICDPNPCENGGICLPGLADGSFSCECPDGFTDPNCSSVVEVASDEEEPTSAGPCTPNPCHNGGTCEISEAYRGDTFIGYVCKCPRGFNGIHCQHNINECEVEPCKNGGICTDLVANYSCECPGEFMGRNCQYKCSGPLGIEGGIISNQQITASSTHRALFGLQKWYPYYARLNKKGLINAWTAAENDRWPWIQINLQRKMRVTGVITQGAKRIGSPEYIKSYKIAYSNDGKTWAMYKVKGTNEDMVFRGNIDNNTPYANSFTPPIKAQYVRLYPQVCRRHCTLRMELLGCELSGCSEPLGMKSGHIQDYQITASSIFRTLNMDMFTWEPRKARLDKQGKVNAWTSGHNDQSQWLQVDLLVPTKVTGIITQGAKDFGHVQFVGSYKLAYSNDGEHWTVYQDEKQRKDKVFQGNFDNDTHRKNVIDPPIYARHIRILPWSWYGRITLRSELLGCTEEE

SEQ ID NO: 2 - protein, 470 aa, Homo sapiens
MKRSVAVWLLVGLSLGVPQFGKGDICDPNPCENGGICLPGLADGSFSCECPDGFTDPNCSSVVEVGPCTPNPCHNGGTCEISEAYRGDTFIGYVCKCPRGFNGIHCQHNINECEVEPCKNGGICTDLVANYSCECPGEFMGRNCQYKCSGPLGIEGGIISNQQITASSTHRALFGLQKWYPYYARLNKKGLINAWTAAENDRWPWIQINLQRKMRVTGVITQGAKRIGSPEYIKSYKIAYSNDGKTWAMYKVKGTNEDMVFRGNIDNNTPYANSFTPPIKAQYVRLYPQVCRRHCTLRMELLGCELSGCSEPLGMKSGHIQDYQITASSIFRTLNMDMFTWEPRKARLDKQGKVNAWTSGHNDQSQWLQVDLLVPTKVTGIITQGAKDFGHVQFVGSYKLAYSNDGEHWTVYQDEKQRKDKVFQGNFDNDTHRKNVIDPPIYARHIRILPWSWYGRITLRSELLGCTEEE

SEQ ID NO: 3 - RNA, 4814 nt, Homo sapiens
  source 1..4814: mol_type = mRNA
acacgcacgccgcctctgtttgtacacagtgcgctcccggcggcccgctcgctcccctccagctcacgcttcattgttctccaagtcagaagccccgcagccgccgcgcggagaacagcgacagccgagcgcccggtccgcctgtctgccggtgggtctgcctgcccgcgcagcagacccggggcggccgcgggagcccgcgccccgcccgccgcgcctctgccgggacccacccgcagcggagggctgagcccgccggcggctccccggagctcacccacctccgcgcgccggagcgcaggcaaaaggggaggaaaggctcctctctttagtcaccactctcgccctctccaagaatttgtttaacaaagcgctgaggaaagagaacgtcttcttgaattctttagtaggggcggagtctgctgctgccctgcgctgccacctcggctacactgccctccgcgacgacccctgaccagccggggtcacgtccgggagacgggatcatgaagcgctcggtagccgtctggctcttggtcgggctcagcctcggtgtcccccagttcggcaaaggtgatatttgtgatcccaatccatgtgaaaatggaggtatctgtttgccaggattggctgatggttccttttcctgtgagtgtccagatggcttcacagaccccaactgttctagtgttgtggaggttgcatcagatgaagaagaaccaacttcagcaggtccctgcactcctaatccatgccataatggaggaacctgtgaaataagtgaagcataccgaggggatacattcataggctatgtttgtaaatgtccccgaggatttaatgggattcactgtcagcacaacataaatgaatgcgaagttgagccttgcaaaaatggtggaatatgtacagatcttgttgctaactattcctgtgagtgcccaggcgaatttatgggaagaaattgtcaatacaaatgctcaggcccactgggaattgaaggtggaattatatcaaaccagcaaatcacagcttcctctactcaccgagctctttttggactccaaaaatggtatccctactatgcacgtcttaataagaaggggcttataaatgcgtggacagctgcagaaaatgacagatggccgtggattcagataaatttgcaaaggaaaatgagagttactggtgtgattacccaaggagccaagaggattggaagcccagagtatataaaatcctacaaaattgcctacagtaatgatggaaagacttgggcaatgtacaaagtgaaaggcaccaatgaagacatggtgtttcgtggaaacattgataacaacactccatatgctaactctttcacaccccccataaaagctcagtatgtaagactctatccccaagtttgtcgaagacattgcactttgcgaatggaacttcttggctgtgaactgtcgggttgttctgagcctctgggtatgaaatcaggacatatacaagactatcagatcactgcctccagcatcttcagaacgctcaacatggacatgttcacttgggaaccaaggaaagctcggctggacaagcaaggcaaagtgaatgcctggacctctggccacaatgaccagtcacaatggttacaggtggatcttcttgttccaaccaaagtgactggcatcattacacaaggagctaaagattttggtcatgtacagtttgttggctcctacaaactggcttacagcaatgatggagaacactggactgtataccaggatgaaaagcaaagaaaagataaggttttccagggaaattttgacaatgacactcacagaaaaaatgtcatcgaccctcccatctatgcacgacacataagaatccttccttggtcctggtacgggaggatcacattgcggtcagagctgctgggctgcacagaggaggaatgaggggaggctacatttcacaaccctcttccctatttccctaaaagtatctccatggaatgaactgtgcaaaatctgtaggaaactgaatggtttttttttttttttcatgaaaaagtgctcaaattatggtaggcaactaacggtgtttttaagggggtctaagcctgccttttcaatgatttaatttgattttattttatccgtcaaatctcttaagtaacaacacattaagtgtgaattacttttctctcattgtttcctgaattattcgcattggtagaaatatattagggaaagaaagtagccttctttttatagcaagagtaaaaaagtctcaaagtcatcaaataagagcaagagttgatagagcttttacaatcaatactcacctaattctgataaaaggaatactgcaatgttagcaataagtttttttcttctgtaatgactctacgttatcctgtttccctgtgcctaccaaacactgtcaatgtttattacaaaattttaaagaagaatatgtaacatgcagtactgatattataattctcattttactttcattatttctaataagagattatgtgacttctttttcttttagttctattctacattcttaatattgtatattacctgaataattcaatttttttctaattgaatttcctattagttgactaaaagaagtgtcatgtttactcatatatgtagaacatgactgcctatcagtagattgatctgtatttaatattcgttaattaaatctgcagttttatttttgaaggaagccataactatttaatttccaaataattgcttcataaagaatcccatactctcagtttgcacaaaagaacaaaaaatatatatgtctctttaaatttaaatcttcatttagatggtaattacatatccttatatttactttaaaaaatcggcttatttgtttattttataaaaaatttagcaaagaaatattaatatagtgctgcatagtttggccaagcatactcatcatttctttgttcagctccacatttcctgtgaaactaacatcttattgagatttgaaactggtggtagtttcccaggaaggcacaggtggagttatttgtgagaagcaaagtgtttactaatgacaaagtagtaaaccattttcaagatgaaaactgatttctatttattttgcttcaaaggtcctgaaaaaataagcaattatcataacaatttgttattgatactggaggtttcattgacatgtctctcaaattaaagctcacactgcctccataaaagtcttcaacatctaatttataagctttacaagtatttattttataaggcttagacagaattattggagttttaaattaagtgtattggaaaagaaaggatggtatgtgtatgaaatgttaagatcctacgcaacactgctatttttttcctttaatatttgtgctgcataacaaaagccactagactgttactgtcttgtctgtccatgtgttaacagcatttcttaatgatgtatatatggagtggtcttcaatcatagtgaagaatttaaagagaaagtcaattgtattggcatttttaataagaacaaaattagttcgtctaaggggactggctggccacatatttgttccttgcccatatgctttctacttcttgttcttattatgaaattatgaatttgaagcctctgaaatggtgatcagttttcaacatctttcaaaaacaaaattactatttcctccatattgccttttttagataactttaaagttaggattttaaaatatttgtaactggctaaattttaaagtcgtgacaaataattacttaggttcagaaatatacacacacttactctttagccagtttctttcaaggtttactgtcccatcagatatctagccattttcctttgcaaattacataccttcttaagagtgtatttttaagattattacttacgctttatgatgatatagtttttcaaaattatttatagcttcatatgatgttttgtaattttttctattgatacctgttttaaaaatattttccaaggaagttgattaaaattatatttgttaccttttagaaaaagcattgaaatgagtttctcttgctttttcattttccctctgctttatatgctcttcgcaatacatcatgtccaacgggatacctattgttctcatgacacccaaaattgatgagagcaaaggggtcgcaccatatggaaatgttgaaaactattgtaaagtagtattatgaagtagcttttgtgtcattcatgtcgatgacatgaaagtgaagtaaatttattctatgtaaattcacactaaaaccagtacagtaccataagtagaatacatgtaagaatcacctagtcttcactatattgagtaaatataacatgctaattttacaattaatgaaactaaacttttaaacatctccattatatctacatccttttgaaggtatttatcatagttgccaattttaattttaggattgactttctctttctgaatgacttcataaagtttggtgtgaattttgaagacttgggttactaatgattgtatctttgctagtcaacaacttatgaaatatactcaatgcgtctgatgtgtcattaagtgcagaaataactaagacacaaataacctttgcaaaccttcaagctgtgtaatattccaatgttgtttttttctttgtatatatacttatatcacgtaggatgtaaaaccagtatgaccttgtctagtctccaaacttaaaataaacttttgaaaagctgggattcttttgaagcagttgtaattaaacacatttataagaata

SEQ ID NO: 4 - RNA, 4741 nt, Homo sapiens
  source 1..4741: mol_type = mRNA
ctctgtttgtacacagtgcgctcccggcggcccgctcgctcccctccagctcacgcttcattgttctccaagtcagaagccccgcagccgccgcgcggagaacagcgacagccgagcgcccggtccgcctgtctgccggtgggtctgcctgcccgcgcagcagacccggggcggccgcgggagcccgcgccccgcccgccgcgcctctgccgggacccacccgcagcggagggctgagcccgccggcggctccccggagctcacccacctccgcgcgccggagcgcaggcaaaaggggaggaaaggctcctctctttagtcaccactctcgccctctccaagaatttgtttaacaaagcgctgaggaaagagaacgtcttcttgaattctttagtaggggcggagtctgctgctgccctgcgctgccacctcggctacactgccctccgcgacgacccctgaccagccggggtcacgtccgggagacgggatcatgaagcgctcggtagccgtctggctcttggtcgggctcagcctcggtgtcccccagttcggcaaaggtgatatttgtgatcccaatccatgtgaaaatggaggtatctgtttgccaggattggctgatggttccttttcctgtgagtgtccagatggcttcacagaccccaactgttctagtgttgtggaggttggtccctgcactcctaatccatgccataatggaggaacctgtgaaataagtgaagcataccgaggggatacattcataggctatgtttgtaaatgtccccgaggatttaatgggattcactgtcagcacaacataaatgaatgcgaagttgagccttgcaaaaatggtggaatatgtacagatcttgttgctaactattcctgtgagtgcccaggcgaatttatgggaagaaattgtcaatacaaatgctcaggcccactgggaattgaaggtggaattatatcaaaccagcaaatcacagcttcctctactcaccgagctctttttggactccaaaaatggtatccctactatgcacgtcttaataagaaggggcttataaatgcgtggacagctgcagaaaatgacagatggccgtggattcagataaatttgcaaaggaaaatgagagttactggtgtgattacccaaggagccaagaggattggaagcccagagtatataaaatcctacaaaattgcctacagtaatgatggaaagacttgggcaatgtacaaagtgaaaggcaccaatgaagacatggtgtttcgtggaaacattgataacaacactccatatgctaactctttcacaccccccataaaagctcagtatgtaagactctatccccaagtttgtcgaagacattgcactttgcgaatggaacttcttggctgtgaactgtcgggttgttctgagcctctgggtatgaaatcaggacatatacaagactatcagatcactgcctccagcatcttcagaacgctcaacatggacatgttcacttgggaaccaaggaaagctcggctggacaagcaaggcaaagtgaatgcctggacctctggccacaatgaccagtcacaatggttacaggtggatcttcttgttccaaccaaagtgactggcatcattacacaaggagctaaagattttggtcatgtacagtttgttggctcctacaaactggcttacagcaatgatggagaacactggactgtataccaggatgaaaagcaaagaaaagataaggttttccagggaaattttgacaatgacactcacagaaaaaatgtcatcgaccctcccatctatgcacgacacataagaatccttccttggtcctggtacgggaggatcacattgcggtcagagctgctgggctgcacagaggaggaatgaggggaggctacatttcacaaccctcttccctatttccctaaaagtatctccatggaatgaactgtgcaaaatctgtaggaaactgaatggtttttttttttttttcatgaaaaagtgctcaaattatggtaggcaactaacggtgtttttaagggggtctaagcctgccttttcaatgatttaatttgattttattttatccgtcaaatctcttaagtaacaacacattaagtgtgaattacttttctctcattgtttcctgaattattcgcattggtagaaatatattagggaaagaaagtagccttctttttatagcaagagtaaaaaagtctcaaagtcatcaaataagagcaagagttgatagagcttttacaatcaatactcacctaattctgataaaaggaatactgcaatgttagcaataagtttttttcttctgtaatgactctacgttatcctgtttccctgtgcctaccaaacactgtcaatgtttattacaaaattttaaagaagaatatgtaacatgcagtactgatattataattctcattttactttcattatttctaataagagattatgtgacttctttttcttttagttctattctacattcttaatattgtatattacctgaataattcaatttttttctaattgaatttcctattagttgactaaaagaagtgtcatgtttactcatatatgtagaacatgactgcctatcagtagattgatctgtatttaatattcgttaattaaatctgcagttttatttttgaaggaagccataactatttaatttccaaataattgcttcataaagaatcccatactctcagtttgcacaaaagaacaaaaaatatatatgtctctttaaatttaaatcttcatttagatggtaattacatatccttatatttactttaaaaaatcggcttatttgtttattttataaaaaatttagcaaagaaatattaatatagtgctgcatagtttggccaagcatactcatcatttctttgttcagctccacatttcctgtgaaactaacatcttattgagatttgaaactggtggtagtttcccaggaaggcacaggtggagttatttgtgagaagcaaagtgtttactaatgacaaagtagtaaaccattttcaagatgaaaactgatttctatttattttgcttcaaaggtcctgaaaaaataagcaattatcataacaatttgttattgatactggaggtttcattgacatgtctctcaaattaaagctcacactgcctccataaaagtcttcaacatctaatttataagctttacaagtatttattttataaggcttagacagaattattggagttttaaattaagtgtattggaaaagaaaggatggtatgtgtatgaaatgttaagatcctacgcaacactgctatttttttcctttaatatttgtgctgcataacaaaagccactagactgttactgtcttgtctgtccatgtgttaacagcatttcttaatgatgtatatatggagtggtcttcaatcatagtgaagaatttaaagagaaagtcaattgtattggcatttttaataagaacaaaattagttcgtctaaggggactggctggccacatatttgttccttgcccatatgctttctacttcttgttcttattatgaaattatgaatttgaagcctctgaaatggtgatcagttttcaacatctttcaaaaacaaaattactatttcctccatattgccttttttagataactttaaagttaggattttaaaatatttgtaactggctaaattttaaagtcgtgacaaataattacttaggttcagaaatatacacacacttactctttagccagtttctttcaaggtttactgtcccatcagatatctagccattttcctttgcaaattacataccttcttaagagtgtatttttaagattattacttacgctttatgatgatatagtttttcaaaattatttatagcttcatatgatgttttgtaattttttctattgatacctgttttaaaaatattttccaaggaagttgattaaaattatatttgttaccttttagaaaaagcattgaaatgagtttctcttgctttttcattttccctctgctttatatgctcttcgcaatacatcatgtccaacgggatacctattgttctcatgacacccaaaattgatgagagcaaaggggtcgcaccatatggaaatgttgaaaactattgtaaagtagtattatgaagtagcttttgtgtcattcatgtcgatgacatgaaagtgaagtaaatttattctatgtaaattcacactaaaaccagtacagtaccataagtagaatacatgtaagaatcacctagtcttcactatattgagtaaatataacatgctaattttacaattaatgaaactaaacttttaaacatctccattatatctacatccttttgaaggtatttatcatagttgccaattttaattttaggattgactttctctttctgaatgacttcataaagtttggtgtgaattttgaagacttgggttactaatgattgtatctttgctagtcaacaacttatgaaatatactcaatgcgtctgatgtgtcattaagtgcagaaataactaagacacaaataacctttgcaaaccttcaagctgtgtaatattccaatgttgtttttttctttgtatatatacttatatcacgtaggatgtaaaaccagtatgaccttgtctagtctccaaacttaaaataaacttttgaaaagctgggaaaaaaaaaaaa

SEQ ID NO: 5 - RNA, 1443 nt, Homo sapiens
  source 1..1443: mol_type = mRNA
atgaagcgctcggtagccgtctggctcttggtcgggctcagcctcggtgtcccccagttcggcaaaggtgatatttgtgatcccaatccatgtgaaaatggaggtatctgtttgccaggattggctgatggttccttttcctgtgagtgtccagatggcttcacagaccccaactgttctagtgttgtggaggttgcatcagatgaagaagaaccaacttcagcaggtccctgcactcctaatccatgccataatggaggaacctgtgaaataagtgaagcataccgaggggatacattcataggctatgtttgtaaatgtccccgaggatttaatgggattcactgtcagcacaacataaatgaatgcgaagttgagccttgcaaaaatggtggaatatgtacagatcttgttgctaactattcctgtgagtgcccaggcgaatttatgggaagaaattgtcaatacaaatgctcaggcccactgggaattgaaggtggaattatatcaaaccagcaaatcacagcttcctctactcaccgagctctttttggactccaaaaatggtatccctactatgcacgtcttaataagaaggggcttataaatgcgtggacagctgcagaaaatgacagatggccgtggattcagataaatttgcaaaggaaaatgagagttactggtgtgattacccaaggagccaagaggattggaagcccagagtatataaaatcctacaaaattgcctacagtaatgatggaaagacttgggcaatgtacaaagtgaaaggcaccaatgaagacatggtgtttcgtggaaacattgataacaacactccatatgctaactctttcacaccccccataaaagctcagtatgtaagactctatccccaagtttgtcgaagacattgcactttgcgaatggaacttcttggctgtgaactgtcgggttgttctgagcctctgggtatgaaatcaggacatatacaagactatcagatcactgcctccagcatcttcagaacgctcaacatggacatgttcacttgggaaccaaggaaagctcggctggacaagcaaggcaaagtgaatgcctggacctctggccacaatgaccagtcacaatggttacaggtggatcttcttgttccaaccaaagtgactggcatcattacacaaggagctaaagattttggtcatgtacagtttgttggctcctacaaactggcttacagcaatgatggagaacactggactgtataccaggatgaaaagcaaagaaaagataaggttttccagggaaattttgacaatgacactcacagaaaaaatgtcatcgaccctcccatctatgcacgacacataagaatccttccttggtcctggtacgggaggatcacattgcggtcagagctgctgggctgcacagaggaggaatga

SEQ ID NO: 6 - RNA, 1413 nt, Homo sapiens
  source 1..1413: mol_type = mRNA
atgaagcgctcggtagccgtctggctcttggtcgggctcagcctcggtgtcccccagttcggcaaaggtgatatttgtgatcccaatccatgtgaaaatggaggtatctgtttgccaggattggctgatggttccttttcctgtgagtgtccagatggcttcacagaccccaactgttctagtgttgtggaggttggtccctgcactcctaatccatgccataatggaggaacctgtgaaataagtgaagcataccgaggggatacattcataggctatgtttgtaaatgtccccgaggatttaatgggattcactgtcagcacaacataaatgaatgcgaagttgagccttgcaaaaatggtggaatatgtacagatcttgttgctaactattcctgtgagtgcccaggcgaatttatgggaagaaattgtcaatacaaatgctcaggcccactgggaattgaaggtggaattatatcaaaccagcaaatcacagcttcctctactcaccgagctctttttggactccaaaaatggtatccctactatgcacgtcttaataagaaggggcttataaatgcgtggacagctgcagaaaatgacagatggccgtggattcagataaatttgcaaaggaaaatgagagttactggtgtgattacccaaggagccaagaggattggaagcccagagtatataaaatcctacaaaattgcctacagtaatgatggaaagacttgggcaatgtacaaagtgaaaggcaccaatgaagacatggtgtttcgtggaaacattgataacaacactccatatgctaactctttcacaccccccataaaagctcagtatgtaagactctatccccaagtttgtcgaagacattgcactttgcgaatggaacttcttggctgtgaactgtcgggttgttctgagcctctgggtatgaaatcaggacatatacaagactatcagatcactgcctccagcatcttcagaacgctcaacatggacatgttcacttgggaaccaaggaaagctcggctggacaagcaaggcaaagtgaatgcctggacctctggccacaatgaccagtcacaatggttacaggtggatcttcttgttccaaccaaagtgactggcatcattacacaaggagctaaagattttggtcatgtacagtttgttggctcctacaaactggcttacagcaatgatggagaacactggactgtataccaggatgaaaagcaaagaaaagataaggttttccagggaaattttgacaatgacactcacagaaaaaatgtcatcgaccctcccatctatgcacgacacataagaatccttccttggtcctggtacgggaggatcacattgcggtcagagctgctgggctgcacagaggaggaatga

SEQ ID NO: 7 - DNA, 1443 bp, Homo sapiens
  source 1..1443: mol_type = genomic DNA
tcattcctcctctgtgcagcccagcagctctgaccgcaatgtgatcctcccgtaccaggaccaaggaaggattcttatgtgtcgtgcatagatgggagggtcgatgacattttttctgtgagtgtcattgtcaaaatttccctggaaaaccttatcttttctttgcttttcatcctggtatacagtccagtgttctccatcattgctgtaagccagtttgtaggagccaacaaactgtacatgaccaaaatctttagctccttgtgtaatgatgccagtcactttggttggaacaagaagatccacctgtaaccattgtgactggtcattgtggccagaggtccaggcattcactttgccttgcttgtccagccgagctttccttggttcccaagtgaacatgtccatgttgagcgttctgaagatgctggaggcagtgatctgatagtcttgtatatgtcctgatttcatacccagaggctcagaacaacccgacagttcacagccaagaagttccattcgcaaagtgcaatgtcttcgacaaacttggggatagagtcttacatactgagcttttatggggggtgtgaaagagttagcatatggagtgttgttatcaatgtttccacgaaacaccatgtcttcattggtgcctttcactttgtacattgcccaagtctttccatcattactgtaggcaattttgtaggattttatatactctgggcttccaatcctcttggctccttgggtaatcacaccagtaactctcattttcctttgcaaatttatctgaatccacggccatctgtcattttctgcagctgtccacgcatttataagccccttcttattaagacgtgcatagtagggataccatttttggagtccaaaaagagctcggtgagtagaggaagctgtgatttgctggtttgatataattccaccttcaattcccagtgggcctgagcatttgtattgacaatttcttcccataaattcgcctgggcactcacaggaatagttagcaacaagatctgtacatattccaccatttttgcaaggctcaacttcgcattcatttatgttgtgctgacagtgaatcccattaaatcctcggggacatttacaaacatagcctatgaatgtatcccctcggtatgcttcacttatttcacaggttcctccattatggcatggattaggagtgcagggacctgctgaagttggttcttcttcatctgatgcaacctccacaacactagaacagttggggtctgtgaagccatctggacactcacaggaaaaggaaccatcagccaatcctggcaaacagatacctccattttcacatggattgggatcacaaatatcacctttgccgaactgggggacaccgaggctgagcccgaccaagagccagacggctaccgagcgcttcat

SEQ ID NO: 8 - DNA, 1413 bp, Homo sapiens
  source 1..1413: mol_type = genomic DNA
tcattcctcctctgtgcagcccagcagctctgaccgcaatgtgatcctcccgtaccaggaccaaggaaggattcttatgtgtcgtgcatagatgggagggtcgatgacattttttctgtgagtgtcattgtcaaaatttccctggaaaaccttatcttttctttgcttttcatcctggtatacagtccagtgttctccatcattgctgtaagccagtttgtaggagccaacaaactgtacatgaccaaaatctttagctccttgtgtaatgatgccagtcactttggttggaacaagaagatccacctgtaaccattgtgactggtcattgtggccagaggtccaggcattcactttgccttgcttgtccagccgagctttccttggttcccaagtgaacatgtccatgttgagcgttctgaagatgctggaggcagtgatctgatagtcttgtatatgtcctgatttcatacccagaggctcagaacaacccgacagttcacagccaagaagttccattcgcaaagtgcaatgtcttcgacaaacttggggatagagtcttacatactgagcttttatggggggtgtgaaagagttagcatatggagtgttgttatcaatgtttccacgaaacaccatgtcttcattggtgcctttcactttgtacattgcccaagtctttccatcattactgtaggcaattttgtaggattttatatactctgggcttccaatcctcttggctccttgggtaatcacaccagtaactctcattttcctttgcaaatttatctgaatccacggccatctgtcattttctgcagctgtccacgcatttataagccccttcttattaagacgtgcatagtagggataccatttttggagtccaaaaagagctcggtgagtagaggaagctgtgatttgctggtttgatataattccaccttcaattcccagtgggcctgagcatttgtattgacaatttcttcccataaattcgcctgggcactcacaggaatagttagcaacaagatctgtacatattccaccatttttgcaaggctcaacttcgcattcatttatgttgtgctgacagtgaatcccattaaatcctcggggacatttacaaacatagcctatgaatgtatcccctcggtatgcttcacttatttcacaggttcctccattatggcatggattaggagtgcagggaccaacctccacaacactagaacagttggggtctgtgaagccatctggacactcacaggaaaaggaaccatcagccaatcctggcaaacagatacctccattttcacatggattgggatcacaaatatcacctttgccgaactgggggacaccgaggctgagcccgaccaagagccagacggctaccgagcgcttcat

SEQ ID NO: 9 - DNA, 21 bp, synthetic construct
  source 1..21: mol_type = other DNA
agcataccgaggggatacatt

SEQ ID NO: 10 - DNA, 21 bp, synthetic construct
  source 1..21: mol_type = other DNA
caaggctcaacttcgcattca

SEQ ID NO: 11 - DNA, 41 bp, synthetic construct
  source 1..41: mol_type = other DNA
caactttgtataataaagttgagtgcagtggcgggatctcg

SEQ ID NO: 12 - DNA, 43 bp, synthetic construct
  source 1..43: mol_type = other DNA
atgattatctttctagggttaacgacaggggcagaatgaaacc

SEQ ID NO: 13 - DNA, 44 bp, synthetic construct
  source 1..44: mol_type = other DNA
cagactatctttctagggttaactgggtctctgctggttctagc

SEQ ID NO: 14 - DNA, 33 bp, synthetic construct
  source 1..33: mol_type = other DNA
cgtgggatcccatggctgcaggcttcggcgttc

SEQ ID NO: 15 - DNA, 32 bp, synthetic construct
  source 1..32: mol_type = other DNA
ccatgggatcccacgccaccccgtgcctcctg

SEQ ID NO: 16 - DNA, 42 bp, synthetic construct
  source 1..42: mol_type = other DNA
caactttgtatagaaaagttgaggagtttgagacctgcctgg

SEQ ID NO: 17 - DNA, 25 bp, synthetic construct
  source 1..25: mol_type = other DNA
caccggccccccaagacttagcgac

SEQ ID NO: 18 - DNA, 25 bp, synthetic construct
  source 1..25: mol_type = other DNA
aaacgtcgctaagtcttggggggcc

SEQ ID NO: 19 - DNA, 25 bp, synthetic construct
  source 1..25: mol_type = other DNA
caccgcggggtggcgtggggtcgca

SEQ ID NO: 20 - DNA, 25 bp, synthetic construct
  source 1..25: mol_type = other DNA
aaactgcgaccccacgccaccccgc

SEQ ID NO: 21 - DNA, 21 bp, synthetic construct
  source 1..21: mol_type = other DNA
aagaagcatttgtggagcacc

SEQ ID NO: 22 - DNA, 20 bp, synthetic construct
  source 1..20: mol_type = other DNA
tgaatctttattaaactagg

SEQ ID NO: 23 - DNA, 20 bp, synthetic construct
  source 1..20: mol_type = other DNA
aggctgagaacgggaagctt

SEQ ID NO: 24 - DNA, 20 bp, synthetic construct
  source 1..20: mol_type = other DNA
actccacgacgtactcagcg

SEQ ID NO: 25 - DNA, 29 bp, synthetic construct
  source 1..29: mol_type = other DNA
atttctagaatcatgaagcgctcggtagc

SEQ ID NO: 26 - DNA, 29 bp, synthetic construct
  source 1..29: mol_type = other DNA
taagaattctcattcctcctctgtgcagc

SEQ ID NO: 27 - DNA, 22 bp, synthetic construct
  source 1..22: mol_type = other DNA
gggctgcgttgctggtcacatt

SEQ ID NO: 28 - DNA, 22 bp, synthetic construct
  source 1..22: mol_type = other DNA
accccatctccacacacaccac

SEQ ID NO: 29 - DNA, 19 bp, synthetic construct
  source 1..19: mol_type = other DNA
gtggaatatgtacagatct

SEQ ID NO: 30 - DNA, 19 bp, synthetic construct
  source 1..19: mol_type = other DNA
taaggttaagtcgccctcg